European Patent Application EP 4 400 585 A1, published July 17, 2024. Title: タンパク質の翻訳制御システム. Applicant: 国立大学法人東京医科歯科大学. The sequence listing filed with the application follows.

SEQUENCE LISTING (28 sequences)

SEQ ID NO: 1 - skipped

SEQ ID NO: 2 - DNA, 333 bp, Feline calicivirus
  source 1..333: mol_type = other DNA
gccaagggcaagaccaagagcaaagtgggcccctacagaggcagaggcgtggcccttacagacgacgagtatgacgaatggcgcgagcacaacgccaccagaaagctggatctgagcgtggaagatttcctgatgctgcggcacagagccgctctgggagctgatgatgccgacgccgtgaagttcagatcctggtggaacagcagaagccggctggccgacgattacgaggatgtgaccgtgatcggcaaaggcggcgtgaagcacgagaagatccggaccaatactctgagagccgtggacagaggctacgacgtgtccttcgctgaagaa

SEQ ID NO: 3 - protein, 111 aa, Feline calicivirus
AKGKTKSKVGPYRGRGVALTDDEYDEWREHNATRKLDLSVEDFLMLRHRAALGADDADAVKFRSWWNSRSRLADDYEDVTVIGKGGVKHEKIRTNTLRAVDRGYDVSFAEE

SEQ ID NO: 4 - DNA, 348 bp, Enterobacteria phage MS2
  source 1..348: mol_type = other DNA
gcttctaactttactcagttcgttctcgtcgacaatggcggaactggcgacgtgactgtcgccccaagcaacttcgctaacggggtcgctgaatggatcagctctaactcgcgatcacaggcttacaaagtaacctgtagcgttcgtcagagctctgcgcagaatcgcaaatacaccatcaaagtcgaggtgcctaaaggcgcatggaggtcttacttaaatatggaactaaccattccaattttcgccacgaattccgactgcgagcttattgttaaggcaatgcaaggtctcctaaaagatggaaacccgattccctcggccatcgcggccaactccggcatctac

SEQ ID NO: 5 - protein, 116 aa, Enterobacteria phage MS2
ASNFTQFVLVDNGGTGDVTVAPSNFANGVAEWISSNSRSQAYKVTCSVRQSSAQNRKYTIKVEVPKGAWRSYLNMELTIPIFATNSDCELIVKAMQGLLKDGNPIPSAIAANSGIY

SEQ ID NO: 6 - DNA, 357 bp, Archaeoglobus fulgidus
  source 1..357: mol_type = other DNA
atgtacgtgagatttgaggttcctgaggacatgcagaacgaagctctgagtctgctggagaaggttagggagagcggtaaggtaaagaaaggtaccaacgagacgacaaaggctgtggagaggggactggcaaagctcgtttacatcgcagaggatgttgacccgcctgagatcgttgctcatctgcccctcctctgcgaggagaagaatgtgccgtacatttacgttaaaagcaagaacgaccttggaagggctgtgggcattgaggtgccatgcgcttcggcagcgataatcaacgagggagagctgagaaaggagcttggaagccttgtggagaagattaaaggccttcagaag

SEQ ID NO: 7 - protein, 119 aa, Archaeoglobus fulgidus
MYVRFEVPEDMQNEALSLLEKVRESGKVKKGTNETTKAVERGLAKLVYIAEDVDPPEIVAHLPLLCEEKNVPYIYVKSKNDLGRAVGIEVPCASAAIINEGELRKELGSLVEKIKGLQK

SEQ ID NO: 8 - DNA, 627 bp, Homo sapiens
  source 1..627: mol_type = other DNA
atgggctccgtgtccaaccagcagtttgcaggtggctgcgccaaggcggcagaagaggcgcccgaggaggcgccggaggacgcggcccgggcggcggacgagcctcagctgctgcacggtgcgggcatctgtaagtggttcaacgtgcgcatggggttcggcttcctgtccatgaccgcccgcgccggggtcgcgctcgaccccccagtggatgtctttgtgcaccagagtaagctgcacatggaagggttccggagcttgaaggagggtgaggcagtggagttcacctttaagaagtcagccaagggtctggaatccatccgtgtcaccggacctggtggagtattctgtattgggagtgagaggcggccaaaaggaaagagcatgcagaagcgcagatcaaaaggagacaggtgctacaactgtggaggtctagatcatcatgccaaggaatgcaagctgccaccccagcccaagaagtgccacttctgccagagcatcagccatatggtagcctcatgtccgctgaaggcccagcagggccctagtgcacagggaaagccaacctactttcgagaggaagaagaagaaatccacagccctaccctgctcccggaggcacagaat

SEQ ID NO: 9 - protein, 209 aa, Homo sapiens
MGSVSNQQFAGGCAKAAEEAPEEAPEDAARAADEPQLLHGAGICKWFNVRMGFGFLSMTARAGVALDPPVDVFVHQSKLHMEGFRSLKEGEAVEFTFKKSAKGLESIRVTGPGGVFCIGSERRPKGKSMQKRRSKGDRCYNCGGLDHHAKECKLPPQPKKCHFCQSISHMVASCPLKAQQGPSAQGKPTYFREEEEEIHSPTLLPEAQN

SEQ ID NO: 10 - DNA, 687 bp, synthetic construct
  misc_feature 1..687: note = fusion protein (MS2CP and VPg)
  source 1..687: mol_type = other DNA
gcttctaactttactcagttcgttctcgtcgacaatggcggaactggcgacgtgactgtcgccccaagcaacttcgctaacggggtcgctgaatggatcagctctaactcgcgatcacaggcttacaaagtaacctgtagcgttcgtcagagctctgcgcagaatcgcaaatacaccatcaaagtcgaggtgcctaaaggcgcatggaggtcttacttaaatatggaactaaccattccaattttcgccacgaattccgactgcgagcttattgttaaggcaatgcaaggtctcctaaaagatggaaacccgattccctcggccatcgcggccaactccggcatctacggatccgccaagggcaagaccaagagcaaagtgggcccctacagaggcagaggcgtggcccttacagacgacgagtatgacgaatggcgcgagcacaacgccaccagaaagctggatctgagcgtggaagatttcctgatgctgcggcacagagccgctctgggagctgatgatgccgacgccgtgaagttcagatcctggtggaacagcagaagccggctggccgacgattacgaggatgtgaccgtgatcggcaaaggcggcgtgaagcacgagaagatccggaccaatactctgagagccgtggacagaggctacgacgtgtccttcgctgaagaa

SEQ ID NO: 11 - protein, 229 aa, synthetic construct
  REGION 1..229: note = fusion protein (MS2CP and VPg)
ASNFTQFVLVDNGGTGDVTVAPSNFANGVAEWISSNSRSQAYKVTCSVRQSSAQNRKYTIKVEVPKGAWRSYLNMELTIPIFATNSDCELIVKAMQGLLKDGNPIPSAIAANSGIYGSAKGKTKSKVGPYRGRGVALTDDEYDEWREHNATRKLDLSVEDFLMLRHRAALGADDADAVKFRSWWNSRSRLADDYEDVTVIGKGGVKHEKIRTNTLRAVDRGYDVSFAEE

SEQ ID NO: 12 - RNA, 103 nt, synthetic construct
  misc_feature 1..103: note = Off switch 5' UTR
  source 1..103: mol_type = other RNA
aggtcagatccgctagcggatccgggagcaggtgaggatcacccatctgccacgagcgaggtgaggatcacccatctcgctcgtgttcccaccggtcgccacc

SEQ ID NO: 13 - RNA, 76 nt, synthetic construct
  misc_feature 1..76: note = On switch 5' UTR
  source 1..76: mol_type = other RNA
gggcgaattaagagagaaaagaagagtacatgaggattacccatgtaagaagaaatataagacaccggtcgccacc

SEQ ID NO: 14 - protein, 189 aa, synthetic construct
  REGION 1..189: note = Caged eNpu N-Intein
CLSYETEILTVEYGLLPIGKIVEKRIECTVYSVDNNGNIYTQPVAQWHDRGKQKVFEYCLEDGSLIRATKDHKFMTVDGQMLPIKEIFRRKLDLMRVDNLPNGSGGENLYFQGENLYFQGGSGGIEIATEKYLGEQNVYDIGVERDHNFALKNGGYFQGIEIATEKYLGEQNVYDIGVERDHNFALKNG

SEQ ID NO: 15 - protein, 109 aa, synthetic construct
  REGION 1..109: note = Caged Npu C-Intein
GEQEVFEYCLEDGSLIRATKDHKFMTVDGQMLPIDEIFERELDLMRVDNLPNGSGGENLYFQGENLYFQGGSGGIKIATRKYLGKQNVYDIGVERDHNFALKNGFIASN

SEQ ID NO: 16 - DNA, 6512 bp, synthetic construct
  misc_feature 1..6512: note = pcDNA3.1-MS2CP(1-45)-eNpuNcage-Nb113
  source 1..6512: mol_type = other DNA
gacggatcgggagatctcccgatcccctatggtgcactctcagtacaatctgctctgatgccgcatagttaagccagtatctgctccctgcttgtgtgttggaggtcgctgagtagtgcgcgagcaaaatttaagctacaacaaggcaaggcttgaccgacaattgcatgaagaatctgcttagggttaggcgttttgcgctgcttcgcgatgtacgggccagatatacgcgttgacattgattattgactagttattaatagtaatcaattacggggtcattagttcatagcccatatatggagttccgcgttacataacttacggtaaatggcccgcctggctgaccgcccaacgacccccgcccattgacgtcaataatgacgtatgttcccatagtaacgccaatagggactttccattgacgtcaatgggtggagtatttacggtaaactgcccacttggcagtacatcaagtgtatcatatgccaagtacgccccctattgacgtcaatgacggtaaatggcccgcctggcattatgcccagtacatgaccttatgggactttcctacttggcagtacatctacgtattagtcatcgctattaccatggtgatgcggttttggcagtacatcaatgggcgtggatagcggtttgactcacggggatttccaagtctccaccccattgacgtcaatgggagtttgttttggcaccaaaatcaacgggactttccaaaatgtcgtaacaactccgccccattgacgcaaatgggcggtaggcgtgtacggtgggaggtctatataagcagagctctctggctaactagagaacccactgcttactggcttatcgaaattaatacgactcactatagggagacccaagctggctagcgtttaaacttaagcttggtaccgccaccatggcttctaactttactcagttcgttctcgtcgacaatggcggaactggcgacgtgactgtcgccccaagcaacttcgctaacggggtcgctgaatggatcagctctaactcgcgatcacaggcttacaaagtaacctgcctgagctacgagacagagatcctgaccgtggaatacggcctgctgcctatcggcaagatcgtggaaaagcggatcgagtgcaccgtgtacagcgtggacaacaacggcaacatctacacccagcctgtggctcagtggcacgacagaggcaagcagaaggtgttcgagtactgcctggaagatggcagcctgatcagagccaccaaggaccacaagttcatgacagtggacggccagatgctgcccatcaaagagatcttccggcggaagctggacctgatgagagtggacaacctgcctaatggctctggcggcgagaacctgtacttccaaggggaaaatctctactttcaaggcggcagcggcggcatcgagatcgccacagagaagtatctgggcgagcagaacgtgtacgacatcggcgtggaacgggaccacaacttcgccctgaagaacggcggctacttccagggaattgagattgccaccgagaaatacctcggggaacagaatgtgtatgatatcggagtcgagcgcgatcacaattttgccctgaaaaatggcggatcccaggtccagctgcaagagtctggcggaggacttgttcaggctggcggaagcctgagactgagctgtactgccagcggcagaaccttcagcagctatgccatgggctggttcagacagacccctggcaaagaacgcgagttcgtggccgccattacatggggcggaagcacaacactgtacgccgactctgtgaagggcagattcaccatgagccgggacaacgccaagaacaccgtgtacctgcagatgaacagcctgaagccagaggacaccgccgtgtactattgtgccgccgatggcagccagtacagaagcacctacagcttcagagacaagcccgactacggctcttggggccagggaacacaagtgaccgtgtcctctcaccaccaccatcaccataccggtgttccaactgttgattacaaggatgacgacgataagtgataaacccgctgatcagcctcgactgtgccttctagttgccagccatctgttgtttgcccctcccccgtgccttccttgaccctggaaggtgccactcccactgtcctttcctaataaaatgaggaaattgcatcgcattgtctgagtaggtgtcattctattctggggggtggggtggggcaggacagcaagggggaggattgggaagacaatagcaggcatgctggggatgcggtgggctctatggcttctgaggcggaaagaaccagctggggctctagggggtatccccacgcgccctgtagcggcgcattaagcgcggcgggtgtggtggttacgcgcagcgtgaccgctacacttgccagcgccctagcgcccgctcctttcgctttcttcccttcctttctcgccacgttcgccggctttccccgtcaagctctaaatcgggggctccctttagggttccgatttagtgctttacggcacctcgaccccaaaaaacttgattagggtgatggttcacgtagtgggccatcgccctgatagacggtttttcgccctttgacgttggagtccacgttctttaatagtggactcttgttccaaactggaacaacactcaaccctatctcggtctattcttttgatttataagggattttgccgatttcggcctattggttaaaaaatgagctgatttaacaaaaatttaacgcgaattaattctgtggaatgtgtgtcagttagggtgtggaaagtccccaggctccccagcaggcagaagtatgcaaagcatgcatctcaattagtcagcaaccaggtgtggaaagtccccaggctccccagcaggcagaagtatgcaaagcatgcatctcaattagtcagcaaccatagtcccgcccctaactccgcccatcccgcccctaactccgcccagttccgcccattctccgccccatggctgactaattttttttatttatgcagaggccgaggccgcctctgcctctgagctattccagaagtagtgaggaggcttttttggaggcctaggcttttgcaaaaagctcccgggagcttgtatatccattttcggatctgatcaagagacaggatgaggatcgtttcgcatgattgaacaagatggattgcacgcaggttctccggccgcttgggtggagaggctattcggctatgactgggcacaacagacaatcggctgctctgatgccgccgtgttccggctgtcagcgcaggggcgcccggttctttttgtcaagaccgacctgtccggtgccctgaatgaactgcaggacgaggcagcgcggctatcgtggctggccacgacgggcgttccttgcgcagctgtgctcgacgttgtcactgaagcgggaagggactggctgctattgggcgaagtgccggggcaggatctcctgtcatctcaccttgctcctgccgagaaagtatccatcatggctgatgcaatgcggcggctgcatacgcttgatccggctacctgcccattcgaccaccaagcgaaacatcgcatcgagcgagcacgtactcggatggaagccggtcttgtcgatcaggatgatctggacgaagagcatcaggggctcgcgccagccgaactgttcgccaggctcaaggcgcgcatgcccgacggcgaggatctcgtcgtgacccatggcgatgcctgcttgccgaatatcatggtggaaaatggccgcttttctggattcatcgactgtggccggctgggtgtggcggaccgctatcaggacatagcgttggctacccgtgatattgctgaagagcttggcggcgaatgggctgaccgcttcctcgtgctttacggtatcgccgctcccgattcgcagcgcatcgccttctatcgccttcttgacgagttcttctgagcgggactctggggttcgaaatgaccgaccaagcgacgcccaacctgccatcacgagatttcgattccaccgccgccttctatgaaaggttgggcttcggaatcgttttccgggacgccggctggatgatcctccagcgcggggatctcatgctggagttcttcgcccaccccaacttgtttattgcagcttataatggttacaaataaagcaatagcatcacaaatttcacaaataaagcatttttttcactgcattctagttgtggtttgtccaaactcatcaatgtatcttatcatgtctgtataccgtcgacctctagctagagcttggcgtaatcatggtcatagctgtttcctgtgtgaaattgttatccgctcacaattccacacaacatacgagccggaagcataaagtgtaaagcctggggtgcctaatgagtgagctaactcacattaattgcgttgcgctcactgcccgctttccagtcgggaaacctgtcgtgccagctgcattaatgaatcggccaacgcgcggggagaggcggtttgcgtattgggcgctcttccgcttcctcgctcactgactcgctgcgctcggtcgttcggctgcggcgagcggtatcagctcactcaaaggcggtaatacggttatccacagaatcaggggataacgcaggaaagaacatgtgagcaaaaggccagcaaaaggccaggaaccgtaaaaaggccgcgttgctggcgtttttccataggctccgcccccctgacgagcatcacaaaaatcgacgctcaagtcagaggtggcgaaacccgacaggactataaagataccaggcgtttccccctggaagctccctcgtgcgctctcctgttccgaccctgccgcttaccggatacctgtccgcctttctcccttcgggaagcgtggcgctttctcatagctcacgctgtaggtatctcagttcggtgtaggtcgttcgctccaagctgggctgtgtgcacgaaccccccgttcagcccgaccgctgcgccttatccggtaactatcgtcttgagtccaacccggtaagacacgacttatcgccactggcagcagccactggtaacaggattagcagagcgaggtatgtaggcggtgctacagagttcttgaagtggtggcctaactacggctacactagaagaacagtatttggtatctgcgctctgctgaagccagttaccttcggaaaaagagttggtagctcttgatccggcaaacaaaccaccgctggtagcggtggtttttttgtttgcaagcagcagattacgcgcagaaaaaaaggatctcaagaagatcctttgatcttttctacggggtctgacgctcagtggaacgaaaactcacgttaagggattttggtcatgagattatcaaaaaggatcttcacctagatccttttaaattaaaaatgaagttttaaatcaatctaaagtatatatgagtaaacttggtctgacagttaccaatgcttaatcagtgaggcacctatctcagcgatctgtctatttcgttcatccatagttgcctgactccccgtcgtgtagataactacgatacgggagggcttaccatctggccccagtgctgcaatgataccgcgagacccacgctcaccggctccagatttatcagcaataaaccagccagccggaagggccgagcgcagaagtggtcctgcaactttatccgcctccatccagtctattaattgttgccgggaagctagagtaagtagttcgccagttaatagtttgcgcaacgttgttgccattgctacaggcatcgtggtgtcacgctcgtcgtttggtatggcttcattcagctccggttcccaacgatcaaggcgagttacatgatcccccatgttgtgcaaaaaagcggttagctccttcggtcctccgatcgttgtcagaagtaagttggccgcagtgttatcactcatggttatggcagcactgcataattctcttactgtcatgccatccgtaagatgcttttctgtgactggtgagtactcaaccaagtcattctgagaatagtgtatgcggcgaccgagttgctcttgcccggcgtcaatacgggataataccgcgccacatagcagaactttaaaagtgctcatcattggaaaacgttcttcggggcgaaaactctcaaggatcttaccgctgttgagatccagttcgatgtaacccactcgtgcacccaactgatcttcagcatcttttactttcaccagcgtttctgggtgagcaaaaacaggaaggcaaaatgccgcaaaaaagggaataagggcgacacggaaatgttgaatactcatactcttcctttttcaatattattgaagcatttatcagggttattgtctcatgagcggatacatatttgaatgtatttagaaaaataaacaaataggggttccgcgcacatttccccgaaaagtgccacctgacgtc

SEQ ID NO: 17 - DNA, 6659 bp, synthetic construct
  misc_feature 1..6659: note = pcDNA3.1-CA1698-NpuCcage-MS2CP(46-116)-VPg(FCV)
  source 1..6659: mol_type = other DNA
gacggatcgggagatctcccgatcccctatggtgcactctcagtacaatctgctctgatgccgcatagttaagccagtatctgctccctgcttgtgtgttggaggtcgctgagtagtgcgcgagcaaaatttaagctacaacaaggcaaggcttgaccgacaattgcatgaagaatctgcttagggttaggcgttttgcgctgcttcgcgatgtacgggccagatatacgcgttgacattgattattgactagttattaatagtaatcaattacggggtcattagttcatagcccatatatggagttccgcgttacataacttacggtaaatggcccgcctggctgaccgcccaacgacccccgcccattgacgtcaataatgacgtatgttcccatagtaacgccaatagggactttccattgacgtcaatgggtggagtatttacggtaaactgcccacttggcagtacatcaagtgtatcatatgccaagtacgccccctattgacgtcaatgacggtaaatggcccgcctggcattatgcccagtacatgaccttatgggactttcctacttggcagtacatctacgtattagtcatcgctattaccatggtgatgcggttttggcagtacatcaatgggcgtggatagcggtttgactcacggggatttccaagtctccaccccattgacgtcaatgggagtttgttttggcaccaaaatcaacgggactttccaaaatgtcgtaacaactccgccccattgacgcaaatgggcggtaggcgtgtacggtgggaggtctatataagcagagctctctggctaactagagaacccactgcttactggcttatcgaaattaatacgactcactatagggagacccaagctggctagcgtttaaacttaagcttggtaccgccaccatggcccaggtccagctgcaagagtctggcggaggacttgttcaggctggcggaagcctgagactgagctgtaaagccagcggcatcatcttcagcgtgtacaagatgacctggtacagacaggcccctggcaaagagagagagctggttgccctgatcaccaccaacaacaataccatgaccgtggacagcgtgaagggcagattcaccatcagccgggacaacgtgcagaacaccgtgtacctggaaatgaacaatctgaagcccgaggacaccgccgtgtactactgcaacgccaatagaggactggccggacctgcctattggggccagggaacacaagtgaccgtgtcctctcaccaccaccatcaccatggatccggcgaacaagaagtgttcgagtactgcctggaagatggcagcctgatcagagccaccaaggaccacaagttcatgaccgtggacggccagatgctgcccatcgacgagatcttcgagcgcgagctggacctgatgagagtggacaacctgcctaatggctctggcggcgagaacctgtacttccaaggggaaaatctctactttcaaggcggcagcggcggcatcaagatcgccacaagaaagtacctgggcaagcagaacgtgtacgacatcggcgtggaacgggaccacaacttcgccctgaagaacggctttatcgccagcaactgtagcgttcgtcagagctctgcgcagaatcgcaaatacaccatcaaagtcgaggtgcctaaaggcgcatggaggtcttacttaaatatggaactaaccattccaattttcgccacgaattccgactgcgagcttattgttaaggcaatgcaaggtctcctaaaagatggaaacccgattccctcggccatcgcggccaactccggcatctacggatccgccaagggcaagaccaagagcaaagtgggcccctacagaggcagaggcgtggcccttacagacgacgagtatgacgaatggcgcgagcacaacgccaccagaaagctggatctgagcgtggaagatttcctgatgctgcggcacagagccgctctgggagctgatgatgccgacgccgtgaagttcagatcctggtggaacagcagaagccggctggccgacgattacgaggatgtgaccgtgatcggcaaaggcggcgtgaagcacgagaagatccggaccaatactctgagagccgtggacagaggctacgacgtgtccttcgctgaagaaaccggtgttccaactgttgattacaaggatgacgacgataagtgataaacccgctgatcagcctcgactgtgccttctagttgccagccatctgttgtttgcccctcccccgtgccttccttgaccctggaaggtgccactcccactgtcctttcctaataaaatgaggaaattgcatcgcattgtctgagtaggtgtcattctattctggggggtggggtggggcaggacagcaagggggaggattgggaagacaatagcaggcatgctggggatgcggtgggctctatggcttctgaggcggaaagaaccagctggggctctagggggtatccccacgcgccctgtagcggcgcattaagcgcggcgggtgtggtggttacgcgcagcgtgaccgctacacttgccagcgccctagcgcccgctcctttcgctttcttcccttcctttctcgccacgttcgccggctttccccgtcaagctctaaatcgggggctccctttagggttccgatttagtgctttacggcacctcgaccccaaaaaacttgattagggtgatggttcacgtagtgggccatcgccctgatagacggtttttcgccctttgacgttggagtccacgttctttaatagtggactcttgttccaaactggaacaacactcaaccctatctcggtctattcttttgatttataagggattttgccgatttcggcctattggttaaaaaatgagctgatttaacaaaaatttaacgcgaattaattctgtggaatgtgtgtcagttagggtgtggaaagtccccaggctccccagcaggcagaagtatgcaaagcatgcatctcaattagtcagcaaccaggtgtggaaagtccccaggctccccagcaggcagaagtatgcaaagcatgcatctcaattagtcagcaaccatagtcccgcccctaactccgcccatcccgcccctaactccgcccagttccgcccattctccgccccatggctgactaattttttttatttatgcagaggccgaggccgcctctgcctctgagctattccagaagtagtgaggaggcttttttggaggcctaggcttttgcaaaaagctcccgggagcttgtatatccattttcggatctgatcaagagacaggatgaggatcgtttcgcatgattgaacaagatggattgcacgcaggttctccggccgcttgggtggagaggctattcggctatgactgggcacaacagacaatcggctgctctgatgccgccgtgttccggctgtcagcgcaggggcgcccggttctttttgtcaagaccgacctgtccggtgccctgaatgaactgcaggacgaggcagcgcggctatcgtggctggccacgacgggcgttccttgcgcagctgtgctcgacgttgtcactgaagcgggaagggactggctgctattgggcgaagtgccggggcaggatctcctgtcatctcaccttgctcctgccgagaaagtatccatcatggctgatgcaatgcggcggctgcatacgcttgatccggctacctgcccattcgaccaccaagcgaaacatcgcatcgagcgagcacgtactcggatggaagccggtcttgtcgatcaggatgatctggacgaagagcatcaggggctcgcgccagccgaactgttcgccaggctcaaggcgcgcatgcccgacggcgaggatctcgtcgtgacccatggcgatgcctgcttgccgaatatcatggtggaaaatggccgcttttctggattcatcgactgtggccggctgggtgtggcggaccgctatcaggacatagcgttggctacccgtgatattgctgaagagcttggcggcgaatgggctgaccgcttcctcgtgctttacggtatcgccgctcccgattcgcagcgcatcgccttctatcgccttcttgacgagttcttctgagcgggactctggggttcgaaatgaccgaccaagcgacgcccaacctgccatcacgagatttcgattccaccgccgccttctatgaaaggttgggcttcggaatcgttttccgggacgccggctggatgatcctccagcgcggggatctcatgctggagttcttcgcccaccccaacttgtttattgcagcttataatggttacaaataaagcaatagcatcacaaatttcacaaataaagcatttttttcactgcattctagttgtggtttgtccaaactcatcaatgtatcttatcatgtctgtataccgtcgacctctagctagagcttggcgtaatcatggtcatagctgtttcctgtgtgaaattgttatccgctcacaattccacacaacatacgagccggaagcataaagtgtaaagcctggggtgcctaatgagtgagctaactcacattaattgcgttgcgctcactgcccgctttccagtcgggaaacctgtcgtgccagctgcattaatgaatcggccaacgcgcggggagaggcggtttgcgtattgggcgctcttccgcttcctcgctcactgactcgctgcgctcggtcgttcggctgcggcgagcggtatcagctcactcaaaggcggtaatacggttatccacagaatcaggggataacgcaggaaagaacatgtgagcaaaaggccagcaaaaggccaggaaccgtaaaaaggccgcgttgctggcgtttttccataggctccgcccccctgacgagcatcacaaaaatcgacgctcaagtcagaggtggcgaaacccgacaggactataaagataccaggcgtttccccctggaagctccctcgtgcgctctcctgttccgaccctgccgcttaccggatacctgtccgcctttctcccttcgggaagcgtggcgctttctcatagctcacgctgtaggtatctcagttcggtgtaggtcgttcgctccaagctgggctgtgtgcacgaaccccccgttcagcccgaccgctgcgccttatccggtaactatcgtcttgagtccaacccggtaagacacgacttatcgccactggcagcagccactggtaacaggattagcagagcgaggtatgtaggcggtgctacagagttcttgaagtggtggcctaactacggctacactagaagaacagtatttggtatctgcgctctgctgaagccagttaccttcggaaaaagagttggtagctcttgatccggcaaacaaaccaccgctggtagcggtggtttttttgtttgcaagcagcagattacgcgcagaaaaaaaggatctcaagaagatcctttgatcttttctacggggtctgacgctcagtggaacgaaaactcacgttaagggattttggtcatgagattatcaaaaaggatcttcacctagatccttttaaattaaaaatgaagttttaaatcaatctaaagtatatatgagtaaacttggtctgacagttaccaatgcttaatcagtgaggcacctatctcagcgatctgtctatttcgttcatccatagttgcctgactccccgtcgtgtagataactacgatacgggagggcttaccatctggccccagtgctgcaatgataccgcgagacccacgctcaccggctccagatttatcagcaataaaccagccagccggaagggccgagcgcagaagtggtcctgcaactttatccgcctccatccagtctattaattgttgccgggaagctagagtaagtagttcgccagttaatagtttgcgcaacgttgttgccattgctacaggcatcgtggtgtcacgctcgtcgtttggtatggcttcattcagctccggttcccaacgatcaaggcgagttacatgatcccccatgttgtgcaaaaaagcggttagctccttcggtcctccgatcgttgtcagaagtaagttggccgcagtgttatcactcatggttatggcagcactgcataattctcttactgtcatgccatccgtaagatgcttttctgtgactggtgagtactcaaccaagtcattctgagaatagtgtatgcggcgaccgagttgctcttgcccggcgtcaatacgggataataccgcgccacatagcagaactttaaaagtgctcatcattggaaaacgttcttcggggcgaaaactctcaaggatcttaccgctgttgagatccagttcgatgtaacccactcgtgcacccaactgatcttcagcatcttttactttcaccagcgtttctgggtgagcaaaaacaggaaggcaaaatgccgcaaaaaagggaataagggcgacacggaaatgttgaatactcatactcttcctttttcaatattattgaagcatttatcagggttattgtctcatgagcggatacatatttgaatgtatttagaaaaataaacaaataggggttccgcgcacatttccccgaaaagtgccacctgacgtc

SEQ ID NO: 18 - DNA, 4713 bp, synthetic construct
  misc_feature 1..4713: note = pSV40-2xScMS2(C)-Luc2
  source 1..4713: mol_type = other DNA
ggcctaactggccggtacctgagctcgctagcctcgaggatatcagatctgcgcagcaccatggcctgaaataacctctgaaagaggaacttggttaggtaccttctgaggcggaaagaaccagctgtggaatgtgtgtcagttagggtgtggaaagtccccaggctccccagcaggcagaagtatgcaaagcatgcatctcaattagtcagcaaccaggtgtggaaagtccccaggctccccagcaggcagaagtatgcaaagcatgcatctcaattagtcagcaaccatagtcccgcccctaactccgcccatcccgcccctaactccgcccagttccgcccattctccgccccatggctgactaattttttttatttatgcagaggccgaggccgcctcggcctctgagctattccagaagtagtgaggaggcttttttggaggcctaggcttttgcaaaaagcttgggagcaggtgaggatcacccatctgccacgagcgaggtgaggatcacccatctcgctcgtgttcccagcttggcaatccggtactgttggtaaagccaccatggaagatgccaaaaacattaagaagggcccagcgccattctacccactcgaagacgggaccgccggcgagcagctgcacaaagccatgaagcgctacgccctggtgcccggcaccatcgcctttaccgacgcacatatcgaggtggacattacctacgccgagtacttcgagatgagcgttcggctggcagaagctatgaagcgctatgggctgaatacaaaccatcggatcgtggtgtgcagcgagaatagcttgcagttcttcatgcccgtgttgggtgccctgttcatcggtgtggctgtggccccagctaacgacatctacaacgagcgcgagctgctgaacagcatgggcatcagccagcccaccgtcgtattcgtgagcaagaaagggctgcaaaagatcctcaacgtgcaaaagaagctaccgatcatacaaaagatcatcatcatggatagcaagaccgactaccagggcttccaaagcatgtacaccttcgtgacttcccatttgccacccggcttcaacgagtacgacttcgtgcccgagagcttcgaccgggacaaaaccatcgccctgatcatgaacagtagtggcagtaccggattgcccaagggcgtagccctaccgcaccgcaccgcttgtgtccgattcagtcatgcccgcgaccccatcttcggcaaccagatcatccccgacaccgctatcctcagcgtggtgccatttcaccacggcttcggcatgttcaccacgctgggctacttgatctgcggctttcgggtcgtgctcatgtaccgcttcgaggaggagctattcttgcgcagcttgcaagactataagattcaatctgccctgctggtgcccacactatttagcttcttcgctaagagcactctcatcgacaagtacgacctaagcaacttgcacgagatcgccagcggcggggcgccgctcagcaaggaggtaggtgaggccgtggccaaacgcttccacctaccaggcatccgccagggctacggcctgacagaaacaaccagcgccattctgatcacccccgaaggggacgacaagcctggcgcagtaggcaaggtggtgcccttcttcgaggctaaggtggtggacttggacaccggtaagacactgggtgtgaaccagcgcggcgagctgtgcgtccgtggccccatgatcatgagcggctacgttaacaaccccgaggctacaaacgctctcatcgacaaggacggctggctgcacagcggcgacatcgcctactgggacgaggacgagcacttcttcatcgtggaccggctgaagagcctgatcaaatacaagggctaccaggtagccccagccgaactggagagcatcctgctgcaacaccccaacatcttcgacgccggggtcgccggcctgcccgacgacgatgccggcgagctgcccgccgcagtcgtcgtgctggaacacggtaaaaccatgaccgagaaggagatcgtggactatgtggccagccaggttacaaccgccaagaagctgcgcggtggtgttgtgttcgtggacgaggtgcctaaaggactgaccggcaagttggacgcccgcaagatccgcgagattctcattaaggccaagaagggcggcaagatcgccgtgtaataattctagagtcggggcggccggccgcttcgagcagacatgataagatacattgatgagtttggacaaaccacaactagaatgcagtgaaaaaaatgctttatttgtgaaatttgtgatgctattgctttatttgtaaccattataagctgcaataaacaagttaacaacaacaattgcattcattttatgtttcaggttcagggggaggtgtgggaggttttttaaagcaagtaaaacctctacaaatgtggtaaaatcgataaggatccgtcgaccgatgcccttgagagccttcaacccagtcagctccttccggtgggcgcggggcatgactatcgtcgccgcacttatgactgtcttctttatcatgcaactcgtaggacaggtgccggcagcgctcttccgcttcctcgctcactgactcgctgcgctcggtcgttcggctgcggcgagcggtatcagctcactcaaaggcggtaatacggttatccacagaatcaggggataacgcaggaaagaacatgtgagcaaaaggccagcaaaaggccaggaaccgtaaaaaggccgcgttgctggcgtttttccataggctccgcccccctgacgagcatcacaaaaatcgacgctcaagtcagaggtggcgaaacccgacaggactataaagataccaggcgtttccccctggaagctccctcgtgcgctctcctgttccgaccctgccgcttaccggatacctgtccgcctttctcccttcgggaagcgtggcgctttctcatagctcacgctgtaggtatctcagttcggtgtaggtcgttcgctccaagctgggctgtgtgcacgaaccccccgttcagcccgaccgctgcgccttatccggtaactatcgtcttgagtccaacccggtaagacacgacttatcgccactggcagcagccactggtaacaggattagcagagcgaggtatgtaggcggtgctacagagttcttgaagtggtggcctaactacggctacactagaagaacagtatttggtatctgcgctctgctgaagccagttaccttcggaaaaagagttggtagctcttgatccggcaaacaaaccaccgctggtagcggtggtttttttgtttgcaagcagcagattacgcgcagaaaaaaaggatctcaagaagatcctttgatcttttctacggggtctgacgctcagtggaacgaaaactcacgttaagggattttggtcatgagattatcaaaaaggatcttcacctagatccttttaaattaaaaatgaagttttaaatcaatctaaagtatatatgagtaaacttggtctgacagcggccgcaaatgctaaaccactgcagtggttaccagtgcttgatcagtgaggcaccgatctcagcgatctgcctatttcgttcgtccatagtggcctgactccccgtcgtgtagatcactacgattcgtgagggcttaccatcaggccccagcgcagcaatgatgccgcgagagccgcgttcaccggcccccgatttgtcagcaatgaaccagccagcagggagggccgagcgaagaagtggtcctgctactttgtccgcctccatccagtctatgagctgctgtcgtgatgctagagtaagaagttcgccagtgagtagtttccgaagagttgtggccattgctactggcatcgtggtatcacgctcgtcgttcggtatggcttcgttcaactctggttcccagcggtcaagccgggtcacatgatcacccatattatgaagaaatgcagtcagctccttagggcctccgatcgttgtcagaagtaagttggccgcggtgttgtcgctcatggtaatggcagcactacacaattctcttaccgtcatgccatccgtaagatgcttttccgtgaccggcgagtactcaaccaagtcgttttgtgagtagtgtatacggcgaccaagctgctcttgcccggcgtctatacgggacaacaccgcgccacatagcagtactttgaaagtgctcatcatcgggaatcgttcttcggggcggaaagactcaaggatcttgccgctattgagatccagttcgatatagcccactcttgcacccagttgatcttcagcatcttttactttcaccagcgtttcggggtgtgcaaaaacaggcaagcaaaatgccgcaaagaagggaatgagtgcgacacgaaaatgttggatgctcatactcgtcctttttcaatattattgaagcatttatcagggttactagtacgtctctcaaggataagtaagtaatattaaggtacgggaggtattggacaggccgcaataaaatatctttattttcattacatctgtgtgttggttttttgtgtgaatcgatagtactaacatacgctctccatcaaaacaaaacgaaacaaaacaaactagcaaaataggctgtccccagtgcaagtgcaggtgccagaacatttctct

SEQ ID NO: 19 - DNA, 3937 bp, synthetic construct
  misc_feature 1..3937: note = pUTR2-MS2CP(1-45)-eNpuNcage-Nb113
  source 1..3937: mol_type = other DNA
tcgcgcgtttcggtgatgacggtgaaaacctctgacacatgcagctcccggagacggtcacagcttgtctgtaagcggatgccgggagcagacaagcccgtcagggcgcgtcagcgggtgttggcgggtgtcggggctggcttaactatgcggcatcagagcagattgtactgagagtgcaccatatgcggtgtgaaataccgcacagatgcgtaaggagaaaataccgcatcaggcgccattcgccattcaggctgcgcaactgttgggaagggcgatcggtgcgggcctcttcgctattacgccagctggcgaaagggggatgtgctgcaaggcgattaagttgggtaacgccagggttttcccagtcacgacgttgtaaaacgacggccagtgatcctctagggcgaattaagagagaaaagaagagtaagaagaaatataagacaccggtcgccaccatggcttctaactttactcagttcgttctcgtcgacaatggcggaactggcgacgtgactgtcgccccaagcaacttcgctaacggggtcgctgaatggatcagctctaactcgcgatcacaggcttacaaagtaacctgcctgagctacgagacagagatcctgaccgtggaatacggcctgctgcctatcggcaagatcgtggaaaagcggatcgagtgcaccgtgtacagcgtggacaacaacggcaacatctacacccagcctgtggctcagtggcacgacagaggcaagcagaaggtgttcgagtactgcctggaagatggcagcctgatcagagccaccaaggaccacaagttcatgacagtggacggccagatgctgcccatcaaagagatcttccggcggaagctggacctgatgagagtggacaacctgcctaatggctctggcggcgagaacctgtacttccaaggggaaaatctctactttcaaggcggcagcggcggcatcgagatcgccacagagaagtatctgggcgagcagaacgtgtacgacatcggcgtggaacgggaccacaacttcgccctgaagaacggcggctacttccagggaattgagattgccaccgagaaatacctcggggaacagaatgtgtatgatatcggagtcgagcgcgatcacaattttgccctgaaaaatggcggatcccaggtccagctgcaagagtctggcggaggacttgttcaggctggcggaagcctgagactgagctgtactgccagcggcagaaccttcagcagctatgccatgggctggttcagacagacccctggcaaagaacgcgagttcgtggccgccattacatggggcggaagcacaacactgtacgccgactctgtgaagggcagattcaccatgagccgggacaacgccaagaacaccgtgtacctgcagatgaacagcctgaagccagaggacaccgccgtgtactattgtgccgccgatggcagccagtacagaagcacctacagcttcagagacaagcccgactacggctcttggggccagggaacacaagtgaccgtgtcctctcaccaccaccatcaccattgaatctagaccttctgcggggcttgccttctggccatgcccttcttctctcccttgcacctgtacctcttggtctttgaataaagcctgagtaggaaaactagagtcgacctgcaggcatgcaagcttggcgtaatcatggtcatagctgtttcctgtgtgaaattgttatccgctcacaattccacacaacatacgagccggaagcataaagtgtaaagcctggggtgcctaatgagtgagctaactcacattaattgcgttgcgctcactgcccgctttccagtcgggaaacctgtcgtgccagctgcattaatgaatcggccaacgcgcggggagaggcggtttgcgtattgggcgctcttccgcttcctcgctcactgactcgctgcgctcggtcgttcggctgcggcgagcggtatcagctcactcaaaggcggtaatacggttatccacagaatcaggggataacgcaggaaagaacatgtgagcaaaaggccagcaaaaggccaggaaccgtaaaaaggccgcgttgctggcgtttttccataggctccgcccccctgacgagcatcacaaaaatcgacgctcaagtcagaggtggcgaaacccgacaggactataaagataccaggcgtttccccctggaagctccctcgtgcgctctcctgttccgaccctgccgcttaccggatacctgtccgcctttctcccttcgggaagcgtggcgctttctcatagctcacgctgtaggtatctcagttcggtgtaggtcgttcgctccaagctgggctgtgtgcacgaaccccccgttcagcccgaccgctgcgccttatccggtaactatcgtcttgagtccaacccggtaagacacgacttatcgccactggcagcagccactggtaacaggattagcagagcgaggtatgtaggcggtgctacagagttcttgaagtggtggcctaactacggctacactagaagaacagtatttggtatctgcgctctgctgaagccagttaccttcggaaaaagagttggtagctcttgatccggcaaacaaaccaccgctggtagcggtggtttttttgtttgcaagcagcagattacgcgcagaaaaaaaggatctcaagaagatcctttgatcttttctacggggtctgacgctcagtggaacgaaaactcacgttaagggattttggtcatgagattatcaaaaaggatcttcacctagatccttttaaattaaaaatgaagttttaaatcaatctaaagtatatatgagtaaacttggtctgacagttaccaatgcttaatcagtgaggcacctatctcagcgatctgtctatttcgttcatccatagttgcctgactccccgtcgtgtagataactacgatacgggagggcttaccatctggccccagtgctgcaatgataccgcgagacccacgctcaccggctccagatttatcagcaataaaccagccagccggaagggccgagcgcagaagtggtcctgcaactttatccgcctccatccagtctattaattgttgccgggaagctagagtaagtagttcgccagttaatagtttgcgcaacgttgttgccattgctacaggcatcgtggtgtcacgctcgtcgtttggtatggcttcattcagctccggttcccaacgatcaaggcgagttacatgatcccccatgttgtgcaaaaaagcggttagctccttcggtcctccgatcgttgtcagaagtaagttggccgcagtgttatcactcatggttatggcagcactgcataattctcttactgtcatgccatccgtaagatgcttttctgtgactggtgagtactcaaccaagtcattctgagaatagtgtatgcggcgaccgagttgctcttgcccggcgtcaatacgggataataccgcgccacatagcagaactttaaaagtgctcatcattggaaaacgttcttcggggcgaaaactctcaaggatcttaccgctgttgagatccagttcgatgtaacccactcgtgcacccaactgatcttcagcatcttttactttcaccagcgtttctgggtgagcaaaaacaggaaggcaaaatgccgcaaaaaagggaataagggcgacacggaaatgttgaatactcatactcttcctttttcaatattattgaagcatttatcagggttattgtctcatgagcggatacatatttgaatgtatttagaaaaataaacaaataggggttccgcgcacatttccccgaaaagtgccacctgacgtctaagaaaccattattatcatgacattaacctataaaaataggcgtatcacgaggccctttcgtc

SEQ ID NO: 20 - DNA, 4084 bp, synthetic construct
  misc_feature 1..4084: note = pUTR2-CA1698-NpuCcage-MS2CP(46-116)-VPg(FCV)
  source 1..4084: mol_type = other DNA
tcgcgcgtttcggtgatgacggtgaaaacctctgacacatgcagctcccggagacggtcacagcttgtctgtaagcggatgccgggagcagacaagcccgtcagggcgcgtcagcgggtgttggcgggtgtcggggctggcttaactatgcggcatcagagcagattgtactgagagtgcaccatatgcggtgtgaaataccgcacagatgcgtaaggagaaaataccgcatcaggcgccattcgccattcaggctgcgcaactgttgggaagggcgatcggtgcgggcctcttcgctattacgccagctggcgaaagggggatgtgctgcaaggcgattaagttgggtaacgccagggttttcccagtcacgacgttgtaaaacgacggccagtgatcctctagggcgaattaagagagaaaagaagagtaagaagaaatataagacaccggtcgccaccatggcccaggtccagctgcaagagtctggcggaggacttgttcaggctggcggaagcctgagactgagctgtaaagccagcggcatcatcttcagcgtgtacaagatgacctggtacagacaggcccctggcaaagagagagagctggttgccctgatcaccaccaacaacaataccatgaccgtggacagcgtgaagggcagattcaccatcagccgggacaacgtgcagaacaccgtgtacctggaaatgaacaatctgaagcccgaggacaccgccgtgtactactgcaacgccaatagaggactggccggacctgcctattggggccagggaacacaagtgaccgtgtcctctcaccaccaccatcaccatggatccggcgaacaagaagtgttcgagtactgcctggaagatggcagcctgatcagagccaccaaggaccacaagttcatgaccgtggacggccagatgctgcccatcgacgagatcttcgagcgcgagctggacctgatgagagtggacaacctgcctaatggctctggcggcgagaacctgtacttccaaggggaaaatctctactttcaaggcggcagcggcggcatcaagatcgccacaagaaagtacctgggcaagcagaacgtgtacgacatcggcgtggaacgggaccacaacttcgccctgaagaacggctttatcgccagcaactgtagcgttcgtcagagctctgcgcagaatcgcaaatacaccatcaaagtcgaggtgcctaaaggcgcatggaggtcttacttaaatatggaactaaccattccaattttcgccacgaattccgactgcgagcttattgttaaggcaatgcaaggtctcctaaaagatggaaacccgattccctcggccatcgcggccaactccggcatctacggatccgccaagggcaagaccaagagcaaagtgggcccctacagaggcagaggcgtggcccttacagacgacgagtatgacgaatggcgcgagcacaacgccaccagaaagctggatctgagcgtggaagatttcctgatgctgcggcacagagccgctctgggagctgatgatgccgacgccgtgaagttcagatcctggtggaacagcagaagccggctggccgacgattacgaggatgtgaccgtgatcggcaaaggcggcgtgaagcacgagaagatccggaccaatactctgagagccgtggacagaggctacgacgtgtccttcgctgaagaatgaatctagaccttctgcggggcttgccttctggccatgcccttcttctctcccttgcacctgtacctcttggtctttgaataaagcctgagtaggaaaactagagtcgacctgcaggcatgcaagcttggcgtaatcatggtcatagctgtttcctgtgtgaaattgttatccgctcacaattccacacaacatacgagccggaagcataaagtgtaaagcctggggtgcctaatgagtgagctaactcacattaattgcgttgcgctcactgcccgctttccagtcgggaaacctgtcgtgccagctgcattaatgaatcggccaacgcgcggggagaggcggtttgcgtattgggcgctcttccgcttcctcgctcactgactcgctgcgctcggtcgttcggctgcggcgagcggtatcagctcactcaaaggcggtaatacggttatccacagaatcaggggataacgcaggaaagaacatgtgagcaaaaggccagcaaaaggccaggaaccgtaaaaaggccgcgttgctggcgtttttccataggctccgcccccctgacgagcatcacaaaaatcgacgctcaagtcagaggtggcgaaacccgacaggactataaagataccaggcgtttccccctggaagctccctcgtgcgctctcctgttccgaccctgccgcttaccggatacctgtccgcctttctcccttcgggaagcgtggcgctttctcatagctcacgctgtaggtatctcagttcggtgtaggtcgttcgctccaagctgggctgtgtgcacgaaccccccgttcagcccgaccgctgcgccttatccggtaactatcgtcttgagtccaacccggtaagacacgacttatcgccactggcagcagccactggtaacaggattagcagagcgaggtatgtaggcggtgctacagagttcttgaagtggtggcctaactacggctacactagaagaacagtatttggtatctgcgctctgctgaagccagttaccttcggaaaaagagttggtagctcttgatccggcaaacaaaccaccgctggtagcggtggtttttttgtttgcaagcagcagattacgcgcagaaaaaaaggatctcaagaagatcctttgatcttttctacggggtctgacgctcagtggaacgaaaactcacgttaagggattttggtcatgagattatcaaaaaggatcttcacctagatccttttaaattaaaaatgaagttttaaatcaatctaaagtatatatgagtaaacttggtctgacagttaccaatgcttaatcagtgaggcacctatctcagcgatctgtctatttcgttcatccatagttgcctgactccccgtcgtgtagataactacgatacgggagggcttaccatctggccccagtgctgcaatgataccgcgagacccacgctcaccggctccagatttatcagcaataaaccagccagccggaagggccgagcgcagaagtggtcctgcaactttatccgcctccatccagtctattaattgttgccgggaagctagagtaagtagttcgccagttaatagtttgcgcaacgttgttgccattgctacaggcatcgtggtgtcacgctcgtcgtttggtatggcttcattcagctccggttcccaacgatcaaggcgagttacatgatcccccatgttgtgcaaaaaagcggttagctccttcggtcctccgatcgttgtcagaagtaagttggccgcagtgttatcactcatggttatggcagcactgcataattctcttactgtcatgccatccgtaagatgcttttctgtgactggtgagtactcaaccaagtcattctgagaatagtgtatgcggcgaccgagttgctcttgcccggcgtcaatacgggataataccgcgccacatagcagaactttaaaagtgctcatcattggaaaacgttcttcggggcgaaaactctcaaggatcttaccgctgttgagatccagttcgatgtaacccactcgtgcacccaactgatcttcagcatcttttactttcaccagcgtttctgggtgagcaaaaacaggaaggcaaaatgccgcaaaaaagggaataagggcgacacggaaatgttgaatactcatactcttcctttttcaatattattgaagcatttatcagggttattgtctcatgagcggatacatatttgaatgtatttagaaaaataaacaaataggggttccgcgcacatttccccgaaaagtgccacctgacgtctaagaaaccattattatcatgacattaacctataaaaataggcgtatcacgaggccctttcgtc

SEQ ID NO: 21 - DNA, 3916 bp, synthetic construct
  misc_feature 1..3916: note = pUTR2-MS2CP(1-45)-eNpuNcage-Lag16
  source 1..3916: mol_type = other DNA
tcgcgcgtttcggtgatgacggtgaaaacctctgacacatgcagctcccggagacggtcacagcttgtctgtaagcggatgccgggagcagacaagcccgtcagggcgcgtcagcgggtgttggcgggtgtcggggctggcttaactatgcggcatcagagcagattgtactgagagtgcaccatatgcggtgtgaaataccgcacagatgcgtaaggagaaaataccgcatcaggcgccattcgccattcaggctgcgcaactgttgggaagggcgatcggtgcgggcctcttcgctattacgccagctggcgaaagggggatgtgctgcaaggcgattaagttgggtaacgccagggttttcccagtcacgacgttgtaaaacgacggccagtgatcctctagggcgaattaagagagaaaagaagagtaagaagaaatataagacaccggtcgccaccatggcttctaactttactcagttcgttctcgtcgacaatggcggaactggcgacgtgactgtcgccccaagcaacttcgctaacggggtcgctgaatggatcagctctaactcgcgatcacaggcttacaaagtaacctgcctgagctacgagacagagatcctgaccgtggaatacggcctgctgcctatcggcaagatcgtggaaaagcggatcgagtgcaccgtgtacagcgtggacaacaacggcaacatctacacccagcctgtggctcagtggcacgacagaggcaagcagaaggtgttcgagtactgcctggaagatggcagcctgatcagagccaccaaggaccacaagttcatgacagtggacggccagatgctgcccatcaaagagatcttccggcggaagctggacctgatgagagtggacaacctgcctaatggctctggcggcgagaacctgtacttccaaggggaaaatctctactttcaaggcggcagcggcggcatcgagatcgccacagagaagtatctgggcgagcagaacgtgtacgacatcggcgtggaacgggaccacaacttcgccctgaagaacggcggctacttccagggaattgagattgccaccgagaaatacctcggggaacagaatgtgtatgatatcggagtcgagcgcgatcacaattttgccctgaaaaatggcggatccgctcaggtgcagctggtggaatctggtggtagactggtgcaggccggcgatagcctgagactgtcttgtgccgccagcggcagaacctttagcacatctgccatggcctggttcagacaggcccctggcagagaaagggaattcgtggccgccatcacatggaccgtgggcaataccatcctgggcgactctgtgaagggcagattcaccatcagccgggacagagccaagaacaccgtggacctgcagatggacaacctggaacctgaggacaccgccgtgtactactgcagcgccagatctagaggctacgtgctgtccgtgctgagaagcgtggacagctacgattattggggccagggcacccaagtgaccgtgtcttgaatctagaccttctgcggggcttgccttctggccatgcccttcttctctcccttgcacctgtacctcttggtctttgaataaagcctgagtaggaaaactagagtcgacctgcaggcatgcaagcttggcgtaatcatggtcatagctgtttcctgtgtgaaattgttatccgctcacaattccacacaacatacgagccggaagcataaagtgtaaagcctggggtgcctaatgagtgagctaactcacattaattgcgttgcgctcactgcccgctttccagtcgggaaacctgtcgtgccagctgcattaatgaatcggccaacgcgcggggagaggcggtttgcgtattgggcgctcttccgcttcctcgctcactgactcgctgcgctcggtcgttcggctgcggcgagcggtatcagctcactcaaaggcggtaatacggttatccacagaatcaggggataacgcaggaaagaacatgtgagcaaaaggccagcaaaaggccaggaaccgtaaaaaggccgcgttgctggcgtttttccataggctccgcccccctgacgagcatcacaaaaatcgacgctcaagtcagaggtggcgaaacccgacaggactataaagataccaggcgtttccccctggaagctccctcgtgcgctctcctgttccgaccctgccgcttaccggatacctgtccgcctttctcccttcgggaagcgtggcgctttctcatagctcacgctgtaggtatctcagttcggtgtaggtcgttcgctccaagctgggctgtgtgcacgaaccccccgttcagcccgaccgctgcgccttatccggtaactatcgtcttgagtccaacccggtaagacacgacttatcgccactggcagcagccactggtaacaggattagcagagcgaggtatgtaggcggtgctacagagttcttgaagtggtggcctaactacggctacactagaagaacagtatttggtatctgcgctctgctgaagccagttaccttcggaaaaagagttggtagctcttgatccggcaaacaaaccaccgctggtagcggtggtttttttgtttgcaagcagcagattacgcgcagaaaaaaaggatctcaagaagatcctttgatcttttctacggggtctgacgctcagtggaacgaaaactcacgttaagggattttggtcatgagattatcaaaaaggatcttcacctagatccttttaaattaaaaatgaagttttaaatcaatctaaagtatatatgagtaaacttggtctgacagttaccaatgcttaatcagtgaggcacctatctcagcgatctgtctatttcgttcatccatagttgcctgactccccgtcgtgtagataactacgatacgggagggcttaccatctggccccagtgctgcaatgataccgcgagacccacgctcaccggctccagatttatcagcaataaaccagccagccggaagggccgagcgcagaagtggtcctgcaactttatccgcctccatccagtctattaattgttgccgggaagctagagtaagtagttcgccagttaatagtttgcgcaacgttgttgccattgctacaggcatcgtggtgtcacgctcgtcgtttggtatggcttcattcagctccggttcccaacgatcaaggcgagttacatgatcccccatgttgtgcaaaaaagcggttagctccttcggtcctccgatcgttgtcagaagtaagttggccgcagtgttatcactcatggttatggcagcactgcataattctcttactgtcatgccatccgtaagatgcttttctgtgactggtgagtactcaaccaagtcattctgagaatagtgtatgcggcgaccgagttgctcttgcccggcgtcaatacgggataataccgcgccacatagcagaactttaaaagtgctcatcattggaaaacgttcttcggggcgaaaactctcaaggatcttaccgctgttgagatccagttcgatgtaacccactcgtgcacccaactgatcttcagcatcttttactttcaccagcgtttctgggtgagcaaaaacaggaaggcaaaatgccgcaaaaaagggaataagggcgacacggaaatgttgaatactcatactcttcctttttcaatattattgaagcatttatcagggttattgtctcatgagcggatacatatttgaatgtatttagaaaaataaacaaataggggttccgcgcacatttccccgaaaagtgccacctgacgtctaagaaaccattattatcatgacattaacctataaaaataggcgtatcacgaggccctttcgtc

SEQ ID NO: 22 - DNA, 4057 bp, synthetic construct
  misc_feature 1..4057: note = pUTR2-GFPenhancerNb-NpuCcage-MS2CP(46-116)-VPg(FCV)
  source 1..4057: mol_type = other DNA
tcgcgcgtttcggtgatgacggtgaaaacctctgacacatgcagctcccggagacggtcacagcttgtctgtaagcggatgccgggagcagacaagcccgtcagggcgcgtcagcgggtgttggcgggtgtcggggctggcttaactatgcggcatcagagcagattgtactgagagtgcaccatatgcggtgtgaaataccgcacagatgcgtaaggagaaaataccgcatcaggcgccattcgccattcaggctgcgcaactgttgggaagggcgatcggtgcgggcctcttcgctattacgccagctggcgaaagggggatgtgctgcaaggcgattaagttgggtaacgccagggttttcccagtcacgacgttgtaaaacgacggccagtgatcctctagggcgaattaagagagaaaagaagagtaagaagaaatataagacaccggtcgccaccatggctcaggtgcagcttgttgaatctggcggagcactggttcagcctggcggatctctgagactgtcttgtgccgcctctggcttccccgtgaaccggtacagcatgcggtggtatagacaggcccctggcaaagaacgagagtgggtggccggaatgtctagcgctggcgatagaagcagctacgaggacagcgtgaagggcagattcaccatcagcagggacgacgccagaaacaccgtgtacctgcagatgaacagcctgaagcctgaggacaccgccgtgtactactgcaacgtgaacgtgggcttcgagtactggggccagggaacccaagtgaccgtttctggatccggcgaacaagaagtgttcgagtactgcctggaagatggcagcctgatcagagccaccaaggaccacaagttcatgaccgtggacggccagatgctgcccatcgacgagatcttcgagcgcgagctggacctgatgagagtggacaacctgcctaatggctctggcggcgagaacctgtacttccaaggggaaaatctctactttcaaggcggcagcggcggcatcaagatcgccacaagaaagtacctgggcaagcagaacgtgtacgacatcggcgtggaacgggaccacaacttcgccctgaagaacggctttatcgccagcaactgtagcgttcgtcagagctctgcgcagaatcgcaaatacaccatcaaagtcgaggtgcctaaaggcgcatggaggtcttacttaaatatggaactaaccattccaattttcgccacgaattccgactgcgagcttattgttaaggcaatgcaaggtctcctaaaagatggaaacccgattccctcggccatcgcggccaactccggcatctacggatccgccaagggcaagaccaagagcaaagtgggcccctacagaggcagaggcgtggcccttacagacgacgagtatgacgaatggcgcgagcacaacgccaccagaaagctggatctgagcgtggaagatttcctgatgctgcggcacagagccgctctgggagctgatgatgccgacgccgtgaagttcagatcctggtggaacagcagaagccggctggccgacgattacgaggatgtgaccgtgatcggcaaaggcggcgtgaagcacgagaagatccggaccaatactctgagagccgtggacagaggctacgacgtgtccttcgctgaagaatgaatctagaccttctgcggggcttgccttctggccatgcccttcttctctcccttgcacctgtacctcttggtctttgaataaagcctgagtaggaaaactagagtcgacctgcaggcatgcaagcttggcgtaatcatggtcatagctgtttcctgtgtgaaattgttatccgctcacaattccacacaacatacgagccggaagcataaagtgtaaagcctggggtgcctaatgagtgagctaactcacattaattgcgttgcgctcactgcccgctttccagtcgggaaacctgtcgtgccagctgcattaatgaatcggccaacgcgcggggagaggcggtttgcgtattgggcgctcttccgcttcctcgctcactgactcgctgcgctcggtcgttcggctgcggcgagcggtatcagctcactcaaaggcggtaatacggttatccacagaatcaggggataacgcaggaaagaacatgtgagcaaaaggccagcaaaaggccaggaaccgtaaaaaggccgcgttgctggcgtttttccataggctccgcccccctgacgagcatcacaaaaatcgacgctcaagtcagaggtggcgaaacccgacaggactataaagataccaggcgtttccccctggaagctccctcgtgcgctctcctgttccgaccctgccgcttaccggatacctgtccgcctttctcccttcgggaagcgtggcgctttctcatagctcacgctgtaggtatctcagttcggtgtaggtcgttcgctccaagctgggctgtgtgcacgaaccccccgttcagcccgaccgctgcgccttatccggtaactatcgtcttgagtccaacccggtaagacacgacttatcgccactggcagcagccactggtaacaggattagcagagcgaggtatgtaggcggtgctacagagttcttgaagtggtggcctaactacggctacactagaagaacagtatttggtatctgcgctctgctgaagccagttaccttcggaaaaagagttggtagctcttgatccggcaaacaaaccaccgctggtagcggtggtttttttgtttgcaagcagcagattacgcgcagaaaaaaaggatctcaagaagatcctttgatcttttctacggggtctgacgctcagtggaacgaaaactcacgttaagggattttggtcatgagattatcaaaaaggatcttcacctagatccttttaaattaaaaatgaagttttaaatcaatctaaagtatatatgagtaaacttggtctgacagttaccaatgcttaatcagtgaggcacctatctcagcgatctgtctatttcgttcatccatagttgcctgactccccgtcgtgtagataactacgatacgggagggcttaccatctggccccagtgctgcaatgataccgcgagacccacgctcaccggctccagatttatcagcaataaaccagccagccggaagggccgagcgcagaagtggtcctgcaactttatccgcctccatccagtctattaattgttgccgggaagctagagtaagtagttcgccagttaatagtttgcgcaacgttgttgccattgctacaggcatcgtggtgtcacgctcgtcgtttggtatggcttcattcagctccggttcccaacgatcaaggcgagttacatgatcccccatgttgtgcaaaaaagcggttagctccttcggtcctccgatcgttgtcagaagtaagttggccgcagtgttatcactcatggttatggcagcactgcataattctcttactgtcatgccatccgtaagatgcttttctgtgactggtgagtactcaaccaagtcattctgagaatagtgtatgcggcgaccgagttgctcttgcccggcgtcaatacgggataataccgcgccacatagcagaactttaaaagtgctcatcattggaaaacgttcttcggggcgaaaactctcaaggatcttaccgctgttgagatccagttcgatgtaacccactcgtgcacccaactgatcttcagcatcttttactttcaccagcgtttctgggtgagcaaaaacaggaaggcaaaatgccgcaaaaaagggaataagggcgacacggaaatgttgaatactcatactcttcctttttcaatattattgaagcatttatcagggttattgtctcatgagcggatacatatttgaatgtatttagaaaaataaacaaataggggttccgcgcacatttccccgaaaagtgccacctgacgtctaagaaaccattattatcatgacattaacctataaaaataggcgtatcacgaggccctttcgtc

SEQ ID NO: 23 - DNA, 1413 bp, synthetic construct
  misc_feature 1..1413: note = MS2CP(1-45)-eNpuNcage-Nb113 template DNA for in vitrotranscription
  source 1..1413: mol_type = other DNA
cagtgaattgtaatacgactcactataaggcgaattaagagagaaaagaagagtaagaagaaatataagacaccggtcgccaccatggcttctaactttactcagttcgttctcgtcgacaatggcggaactggcgacgtgactgtcgccccaagcaacttcgctaacggggtcgctgaatggatcagctctaactcgcgatcacaggcttacaaagtaacctgcctgagctacgagacagagatcctgaccgtggaatacggcctgctgcctatcggcaagatcgtggaaaagcggatcgagtgcaccgtgtacagcgtggacaacaacggcaacatctacacccagcctgtggctcagtggcacgacagaggcaagcagaaggtgttcgagtactgcctggaagatggcagcctgatcagagccaccaaggaccacaagttcatgacagtggacggccagatgctgcccatcaaagagatcttccggcggaagctggacctgatgagagtggacaacctgcctaatggctctggcggcgagaacctgtacttccaaggggaaaatctctactttcaaggcggcagcggcggcatcgagatcgccacagagaagtatctgggcgagcagaacgtgtacgacatcggcgtggaacgggaccacaacttcgccctgaagaacggcggctacttccagggaattgagattgccaccgagaaatacctcggggaacagaatgtgtatgatatcggagtcgagcgcgatcacaattttgccctgaaaaatggcggatcccaggtccagctgcaagagtctggcggaggacttgttcaggctggcggaagcctgagactgagctgtactgccagcggcagaaccttcagcagctatgccatgggctggttcagacagacccctggcaaagaacgcgagttcgtggccgccattacatggggcggaagcacaacactgtacgccgactctgtgaagggcagattcaccatgagccgggacaacgccaagaacaccgtgtacctgcagatgaacagcctgaagccagaggacaccgccgtgtactattgtgccgccgatggcagccagtacagaagcacctacagcttcagagacaagcccgactacggctcttggggccagggaacacaagtgaccgtgtcctctcaccaccaccatcaccattgaatctagaccttctgcggggcttgccttctggccatgcccttcttctctcccttgcacctgtacctcttggtctttgaataaagcctgagtaggaaaaaaaaaaaaaaaaaaaaaaaaaaaaaaaaaaaaaaaaaaaaaaaaaaaaaaaaaaaaaaaaaaaaaaaaaaaaaaaaaaaaaaaaaaaaaaaaaaaaaaaaaaaaaaaaaaaaaaaa

SEQ ID NO: 24 - DNA, 1560 bp, synthetic construct
  misc_feature 1..1560: note = CA1698-NpuCcage-MS2CP(46-116)-VPg(FCV) template DNA for in vitrotranscription
  source 1..1560: mol_type = other DNA
cagtgaattgtaatacgactcactataaggcgaattaagagagaaaagaagagtaagaagaaatataagacaccggtcgccaccatggcccaggtccagctgcaagagtctggcggaggacttgttcaggctggcggaagcctgagactgagctgtaaagccagcggcatcatcttcagcgtgtacaagatgacctggtacagacaggcccctggcaaagagagagagctggttgccctgatcaccaccaacaacaataccatgaccgtggacagcgtgaagggcagattcaccatcagccgggacaacgtgcagaacaccgtgtacctggaaatgaacaatctgaagcccgaggacaccgccgtgtactactgcaacgccaatagaggactggccggacctgcctattggggccagggaacacaagtgaccgtgtcctctcaccaccaccatcaccatggatccggcgaacaagaagtgttcgagtactgcctggaagatggcagcctgatcagagccaccaaggaccacaagttcatgaccgtggacggccagatgctgcccatcgacgagatcttcgagcgcgagctggacctgatgagagtggacaacctgcctaatggctctggcggcgagaacctgtacttccaaggggaaaatctctactttcaaggcggcagcggcggcatcaagatcgccacaagaaagtacctgggcaagcagaacgtgtacgacatcggcgtggaacgggaccacaacttcgccctgaagaacggctttatcgccagcaactgtagcgttcgtcagagctctgcgcagaatcgcaaatacaccatcaaagtcgaggtgcctaaaggcgcatggaggtcttacttaaatatggaactaaccattccaattttcgccacgaattccgactgcgagcttattgttaaggcaatgcaaggtctcctaaaagatggaaacccgattccctcggccatcgcggccaactccggcatctacggatccgccaagggcaagaccaagagcaaagtgggcccctacagaggcagaggcgtggcccttacagacgacgagtatgacgaatggcgcgagcacaacgccaccagaaagctggatctgagcgtggaagatttcctgatgctgcggcacagagccgctctgggagctgatgatgccgacgccgtgaagttcagatcctggtggaacagcagaagccggctggccgacgattacgaggatgtgaccgtgatcggcaaaggcggcgtgaagcacgagaagatccggaccaatactctgagagccgtggacagaggctacgacgtgtccttcgctgaagaatgaatctagaccttctgcggggcttgccttctggccatgcccttcttctctcccttgcacctgtacctcttggtctttgaataaagcctgagtaggaaaaaaaaaaaaaaaaaaaaaaaaaaaaaaaaaaaaaaaaaaaaaaaaaaaaaaaaaaaaaaaaaaaaaaaaaaaaaaaaaaaaaaaaaaaaaaaaaaaaaaaaaaaaaaaaaaaaaaaa

SEQ ID NO: 25 - DNA, 1392 bp, synthetic construct
  misc_feature 1..1392: note = MS2CP(1-45)-eNpuNcage-Lag16 template DNA for in vitrotranscription
  source 1..1392: mol_type = other DNA
cagtgaattgtaatacgactcactataaggcgaattaagagagaaaagaagagtaagaagaaatataagacaccggtcgccaccatggcttctaactttactcagttcgttctcgtcgacaatggcggaactggcgacgtgactgtcgccccaagcaacttcgctaacggggtcgctgaatggatcagctctaactcgcgatcacaggcttacaaagtaacctgcctgagctacgagacagagatcctgaccgtggaatacggcctgctgcctatcggcaagatcgtggaaaagcggatcgagtgcaccgtgtacagcgtggacaacaacggcaacatctacacccagcctgtggctcagtggcacgacagaggcaagcagaaggtgttcgagtactgcctggaagatggcagcctgatcagagccaccaaggaccacaagttcatgacagtggacggccagatgctgcccatcaaagagatcttccggcggaagctggacctgatgagagtggacaacctgcctaatggctctggcggcgagaacctgtacttccaaggggaaaatctctactttcaaggcggcagcggcggcatcgagatcgccacagagaagtatctgggcgagcagaacgtgtacgacatcggcgtggaacgggaccacaacttcgccctgaagaacggcggctacttccagggaattgagattgccaccgagaaatacctcggggaacagaatgtgtatgatatcggagtcgagcgcgatcacaattttgccctgaaaaatggcggatccgctcaggtgcagctggtggaatctggtggtagactggtgcaggccggcgatagcctgagactgtcttgtgccgccagcggcagaacctttagcacatctgccatggcctggttcagacaggcccctggcagagaaagggaattcgtggccgccatcacatggaccgtgggcaataccatcctgggcgactctgtgaagggcagattcaccatcagccgggacagagccaagaacaccgtggacctgcagatggacaacctggaacctgaggacaccgccgtgtactactgcagcgccagatctagaggctacgtgctgtccgtgctgagaagcgtggacagctacgattattggggccagggcacccaagtgaccgtgtcttgaatctagaccttctgcggggcttgccttctggccatgcccttcttctctcccttgcacctgtacctcttggtctttgaataaagcctgagtaggaaaaaaaaaaaaaaaaaaaaaaaaaaaaaaaaaaaaaaaaaaaaaaaaaaaaaaaaaaaaaaaaaaaaaaaaaaaaaaaaaaaaaaaaaaaaaaaaaaaaaaaaaaaaaaaaaaaaaaaa

SEQ ID NO: 26 - DNA, 1533 bp, synthetic construct
  misc_feature 1..1533: note = GFPenhancerNb-NpuCcage-MS2CP(46-116)-VPg(FCV) template DNA for invitro transcription
  source 1..1533: mol_type = other DNA
cagtgaattgtaatacgactcactataaggcgaattaagagagaaaagaagagtaagaagaaatataagacaccggtcgccaccatggctcaggtgcagcttgttgaatctggcggagcactggttcagcctggcggatctctgagactgtcttgtgccgcctctggcttccccgtgaaccggtacagcatgcggtggtatagacaggcccctggcaaagaacgagagtgggtggccggaatgtctagcgctggcgatagaagcagctacgaggacagcgtgaagggcagattcaccatcagcagggacgacgccagaaacaccgtgtacctgcagatgaacagcctgaagcctgaggacaccgccgtgtactactgcaacgtgaacgtgggcttcgagtactggggccagggaacccaagtgaccgtttctggatccggcgaacaagaagtgttcgagtactgcctggaagatggcagcctgatcagagccaccaaggaccacaagttcatgaccgtggacggccagatgctgcccatcgacgagatcttcgagcgcgagctggacctgatgagagtggacaacctgcctaatggctctggcggcgagaacctgtacttccaaggggaaaatctctactttcaaggcggcagcggcggcatcaagatcgccacaagaaagtacctgggcaagcagaacgtgtacgacatcggcgtggaacgggaccacaacttcgccctgaagaacggctttatcgccagcaactgtagcgttcgtcagagctctgcgcagaatcgcaaatacaccatcaaagtcgaggtgcctaaaggcgcatggaggtcttacttaaatatggaactaaccattccaattttcgccacgaattccgactgcgagcttattgttaaggcaatgcaaggtctcctaaaagatggaaacccgattccctcggccatcgcggccaactccggcatctacggatccgccaagggcaagaccaagagcaaagtgggcccctacagaggcagaggcgtggcccttacagacgacgagtatgacgaatggcgcgagcacaacgccaccagaaagctggatctgagcgtggaagatttcctgatgctgcggcacagagccgctctgggagctgatgatgccgacgccgtgaagttcagatcctggtggaacagcagaagccggctggccgacgattacgaggatgtgaccgtgatcggcaaaggcggcgtgaagcacgagaagatccggaccaatactctgagagccgtggacagaggctacgacgtgtccttcgctgaagaatgaatctagaccttctgcggggcttgccttctggccatgcccttcttctctcccttgcacctgtacctcttggtctttgaataaagcctgagtaggaaaaaaaaaaaaaaaaaaaaaaaaaaaaaaaaaaaaaaaaaaaaaaaaaaaaaaaaaaaaaaaaaaaaaaaaaaaaaaaaaaaaaaaaaaaaaaaaaaaaaaaaaaaaaaaaaaaaaaaa

SEQ ID NO: 27 - DNA, 819 bp, synthetic construct
  misc_feature 1..819: note = eDHFR-DYKtag template DNA for in vitro transcription
  source 1..819: mol_type = other DNA
cagtgaattgtaatacgactcactataaggcgaattaagagagaaaagaagagtaagaagaaatataagacaccggtcgccaccatgatcagtctgattgcggcgttagcggtagatcgcgttatcggcatggaaaacgccatgccgtggaacctgcctgccgatctcgcctggtttaaacgcaacaccttaaataaacccgtgattatgggccgccatacctgggaatcaatcggtcgtccgttgccaggacgcaaaaatattatcctcagcagtcaaccgggtacggacgatcgcgtaacgtgggtgaagtcggtggatgaagccatcgcggcgtgtggtgacgtaccagaaatcatggtgattggcggcggtcgcgtttatgaacagttcttgccaaaagcgcaaaaactgtatctgacgcatatcgacgcagaagtggaaggcgacacccatttcccggattacgagccggatgactgggaatcggtattcagcgaattccacgatgctgatgcgcagaactctcacagctattgctttgagattctggagcggcggaccggtgttccaactgttgattacaaggatgacgacgataagtgaatctagaccttctgcggggcttgccttctggccatgcccttcttctctcccttgcacctgtacctcttggtctttgaataaagcctgagtaggaaaaaaaaaaaaaaaaaaaaaaaaaaaaaaaaaaaaaaaaaaaaaaaaaaaaaaaaaaaaaaaaaaaaaaaaaaaaaaaaaaaaaaaaaaaaaaaaaaaaaaaaaaaaaaaaaaaaaaaa

SEQ ID NO: 28 - DNA, 1017 bp, synthetic construct
  misc_feature 1..1017: note = EGFP template DNA for in vitro transcription
  source 1..1017: mol_type = other DNA
cagtgaattgtaatacgactcactataaggcgaattaagagagaaaagaagagtaagaagaaatataagacaccggtcgccaccatggtgagcaagggcgaggagctgttcaccggggtggtgcccatcctggtcgagctggacggcgacgtaaacggccacaagttcagcgtgtccggcgagggcgagggcgatgccacctacggcaagctgaccctgaagttcatctgcaccaccggcaagctgcccgtgccctggcccaccctcgtgaccaccctgacctacggcgtgcagtgcttcagccgctaccccgaccacatgaagcagcacgacttcttcaagtccgccatgcccgaaggctacgtccaggagcgcaccatcttcttcaaggacgacggcaactacaagacccgcgccgaggtgaagttcgagggcgacaccctggtgaaccgcatcgagctgaagggcatcgacttcaaggaggacggcaacatcctggggcacaagctggagtacaactacaacagccacaacgtctatatcatggccgacaagcagaagaacggcatcaaggtgaacttcaagatccgccacaacatcgaggacggcagcgtgcagctcgccgaccactaccagcagaacacccccatcggcgacggccccgtgctgctgcccgacaaccactacctgagcacccagtccgccctgagcaaagaccccaacgagaagcgcgatcacatggtcctgctggagttcgtgaccgccgccgggatcactctcggcatggacgagctgtacaagtaaatctagaccttctgcggggcttgccttctggccatgcccttcttctctcccttgcacctgtacctcttggtctttgaataaagcctgagtaggaaaaaaaaaaaaaaaaaaaaaaaaaaaaaaaaaaaaaaaaaaaaaaaaaaaaaaaaaaaaaaaaaaaaaaaaaaaaaaaaaaaaaaaaaaaaaaaaaaaaaaaaaaaaaaaaaaaaaaaa